European Patent Specification EP 3 414 573 B1, published November 8, 2023. Title: NOVEL ANTI-LAM AND ANTI-PIM6 MONOCLONAL ANTIBODIES FOR DIAGNOSIS AND TREATMENT OF MYCOBACTERIUM TUBERCULOSIS INFECTIONS. Applicant: Rutgers, The State University of New Jersey Pinter, Abraham Patel, Deendayal Choudhary, Alok. The sequence listing filed with the application follows.

SEQUENCE LISTING (50 sequences)

SEQ ID NO: 1 - protein, 6 aa, HOMO SAPIENS
RSIRSA

SEQ ID NO: 2 - protein, 3 aa, HOMO SAPIENS
GAS

SEQ ID NO: 3 - protein, 9 aa, HOMO SAPIENS
QQYDFWYTF

SEQ ID NO: 4 - protein, 8 aa, HOMO SAPIENS
GFNFEDFG

SEQ ID NO: 5 - protein, 8 aa, HOMO SAPIENS
ISWNGANI

SEQ ID NO: 6 - protein, 13 aa, HOMO SAPIENS
IDWYRDDYYKMDV

SEQ ID NO: 7 - protein, 6 aa, HOMO SAPIENS
QSINSN

SEQ ID NO: 8 - protein, 3 aa, HOMO SAPIENS
KAS

SEQ ID NO: 9 - protein, 9 aa, HOMO SAPIENS
QQYKAFKTF

SEQ ID NO: 10 - protein, 8 aa, HOMO SAPIENS
GGSFSGYY

SEQ ID NO: 11 - protein, 13 aa, HOMO SAPIENS
FDLGGSITHSRGT

SEQ ID NO: 12 - protein, 13 aa, HOMO SAPIENS
RGLAMGGTKEFDS

SEQ ID NO: 13 - protein, 12 aa, HOMO SAPIENS
QNVLDSANNRNY

SEQ ID NO: 14 - protein, 3 aa, HOMO SAPIENS
WAS

SEQ ID NO: 15 - protein, 9 aa, HOMO SAPIENS
TQYHRLPHT

SEQ ID NO: 16 - protein, 9 aa, HOMO SAPIENS
GGSINTNNW

SEQ ID NO: 17 - protein, 7 aa, HOMO SAPIENS
IHRHGDT

SEQ ID NO: 18 - protein, 15 aa, HOMO SAPIENS
CPLGYCSGDDCHRVA

SEQ ID NO: 19 - protein, 5 aa, HOMO SAPIENS
GGSGG

SEQ ID NO: 20 - skipped

SEQ ID NO: 21 - protein, 96 aa, HOMO SAPIENS
QVQLLESGGGVVRPGGSLRLSCAASGFNFEDFGMSWVRQAPGKGLEWVSSISWNGANIGYVDSVKGRFTISRDNAKNSLYLQMNSLRAEDTALYYC

SEQ ID NO: 22 - protein, 96 aa, HOMO SAPIENS
EVQLVESGGGVVRPGGSLRLSCAASGFTFDDYGMSWVRQAPGKGLEWVSGINWNGGSTGYADSVKGRFTISRDNAKNSLYLQMNSLRAEDTALYHC

SEQ ID NO: 23 - protein, 14 aa, HOMO SAPIENS
AIDWYRDDYYKMDV

SEQ ID NO: 24 - protein, 88 aa, HOMO SAPIENS
EIVMTQSPATLSVSPGERATLSCRASRSIRSALAWYQHKPGQAPRLLIFGASTRATGIPARFSGSGSGTDFTLTVSSIRSEDSAVYYC

SEQ ID NO: 25 - protein, 88 aa, HOMO SAPIENS
EIVMTQSPATLSVSPGERATLSCRASQSVSSNLAWYQQKPGQAPRLLIYGASTRATGIPARFSGSGSGTEFTLTISSLQSEDFAVYYC

SEQ ID NO: 26 - protein, 8 aa, HOMO SAPIENS
QQYDFWYT

SEQ ID NO: 27 - protein, 101 aa, HOMO SAPIENS
QVQLQQWGAGLLKPSETLSLTCAVYGGSFSGYYWSWIRQSPETGLEWLGEFDLGGSITHSRGTNYNPSLKSRVTISGDTSKNQFSLKLTSVTAADTAVYYC

SEQ ID NO: 28 - protein, 95 aa, HOMO SAPIENS
QVQLQQWGAGLLKPSETLSLTCAVYGGSFSGYYWSWIRQPPGKGLEWIGEINHSGSTNYNPSLKSRVTISVDTSKNQFSLKLSSVTAADTAVYYC

SEQ ID NO: 29 - protein, 14 aa, HOMO SAPIENS
ARGLAMGGTKEFDS

SEQ ID NO: 30 - protein, 88 aa, HOMO SAPIENS
DIQMTQSPDSLSASVGDRITITCRASQSINSNLAWYQQKPGKAPKLLIYKASDLESGVPSRFSGSGSGTEFTLTISSLQPDDFATYYC

SEQ ID NO: 31 - protein, 88 aa, HOMO SAPIENS
DIQMTQSPSTLSASVGDRVTITCRASQSISSWLAWYQQKPGKAPKLLIYKASSLESGVPSRFSGSGSGTEFTLTISSLQPDDFATYYC

SEQ ID NO: 32 - protein, 8 aa, HOMO SAPIENS
QQYKAFKT

SEQ ID NO: 33 - protein, 96 aa, HOMO SAPIENS
EVQLLESGPGLVRPWGTLSLTCAVSGGSINTNNWWSWVRQSPGKGLEWIGEIHRHGDTNYNPSLKRRVSISMDESMNQFSLRLISVTAADTAVYYC

SEQ ID NO: 34 - protein, 96 aa, HOMO SAPIENS
QVQLQESGPGLVKPSGTLSLTCAVSGGSISSSNWWSWVRQPPGKGLEWIGEIYHSGSTNYNPSLKSRVTISVDKSKNQFSLKLSSVTAADTAVYYC

SEQ ID NO: 35 - skipped

SEQ ID NO: 36 - protein, 94 aa, HOMO SAPIENS
DIQMTQSPSSLSVSLGERATINCKSSQNVLDSANNRNYFGWYQQKPGQPPKLLISWASTRESGVPDRFSGSGSGTDFTLIISGLQVEDVAVYYC

SEQ ID NO: 37 - protein, 94 aa, HOMO SAPIENS
DIVMTQSPDSLAVSLGERATINCKSSQSVLYSSNNKNYLAWYQQKPGQPPKLLIYWASTRESGVPDRFSGSGSGTDFTLTISSLQAEDVAVYYC

SEQ ID NO: 38 - skipped

SEQ ID NO: 39 - DNA, 1356 bp, homo sapiens
caagtgcagctgttggagtctgggggaggtgtggtacggccgggggggtccctgagactctcctgtgcagcctctggattcaactttgaagattttggcatgagctgggtccgccaagctccagggaaggggctggagtgggtctctagtattagttggaatggtgctaatataggctatgtagactctgtgaagggccgattcaccatctccagagacaacgccaagaactccctatatctgcaaatgaacagtctgagagccgaggacacggccttatattactgtgcgatagactggtacagagacgactactacaagatggacgtctggggcaaagggaccacggtcaccgtctcctcagcctcgaccaagggcccatcggtcttcccgctagcgccctcctccaagagcacctctgggggcacagcggccctgggctgcctggtcaaggactacttccccgaacctgtgacggtctcgtggaactcaggcgccctgaccagcggcgtgcacaccttcccggctgtcctacagtcctcaggactctactccctcagcagcgtggtgaccgtgccctccagcagcttgggcacccagacctacatctgcaacgtgaatcacaagcccagcaacaccaaggtggacaagaaagttgagcccaaatcttgtgacaaaactcacacatgcccaccgtgcccagcacctgaactcctggggggaccgtcagtcttcctcttccccccaaaacccaaggacaccctcatgatctcccggacccctgaggtcacatgcgtggtggtggacgtgagccacgaagaccctgaggtcaagttcaactggtacgtggacggcgtggaggtgcataatgccaagacaaagccgcgggaggagcagtacaacagcacgtaccgtgtggtcagcgtcctcaccgtcctgcaccaggactggctgaatggcaaggagtacaagtgcaaggtctccaacaaagccctcccagcccccatcgagaaaaccatctccaaagccaaagggcagccccgagaaccacaggtgtacaccctgcccccatcccgggatgagctgaccaagaaccaggtcagcctgacctgcctggtcaaaggcttctatcccagcgacatcgccgtggagtgggagagcaatgggcagccggagaacaactacaagaccacgcctcccgtgctggactccgacggctccttcttcctctacagcaagctcaccgtggacaagagcaggtggcagcaggggaacgtcttctcatgctccgtgatgcatgaggctctgcacaaccactacacgcagaagagcctctccctgtctccgggtaaatga

SEQ ID NO: 40 - protein, 451 aa, HOMO SAPIENS
QVQLLESGGGVVRPGGSLRLSCAASGFNFEDFGMSWVRQAPGKGLEWVSSISWNGANIGYVDSVKGRFTISRDNAKNSLYLQMNSLRAEDTALYYCAIDWYRDDYYKMDVWGKGTTVTVSSASTKGPSVFPLAPSSKSTSGGTAALGCLVKDYFPEPVTVSWNSGALTSGVHTFPAVLQSSGLYSLSSVVTVPSSSLGTQTYICNVNHKPSNTKVDKKVEPKSCDKTHTCPPCPAPELLGGPSVFLFPPKPKDTLMISRTPEVTCVVVDVSHEDPEVKFNWYVDGVEVHNAKTKPREEQYNSTYRVVSVLTVLHQDWLNGKEYKCKVSNKALPAPIEKTISKAKGQPREPQVYTLPPSRDELTKNQVSLTCLVKGFYPSDIAVEWESNGQPENNYKTTPPVLDSDGSFFLYSKLTVDKSRWQQGNVFSCSVMHEALHNHYTQKSLSLSPGK

SEQ ID NO: 41 - DNA, 642 bp, HOMO SAPIENS
gaaatagtgatgacgcagtctccagccaccctgtctgtctctccaggggaaagagccaccctctcctgcagggccagtcggagtattcgcagcgccttagcctggtaccagcacaaacctggccaggctcccaggctcctcatctttggtgcatccaccagggccactggtatcccagccaggttcagtggcagtgggtctgggacagacttcactctcaccgtcagcagcatacggtctgaggattctgcagtttattactgtcagcagtatgatttctggtacacttttggccaggggaccaagctggagatcaaacgaactgtggctgcaccatctgtcttcatcttcccgccatctgatgagcagttgaaatctggaactgcctctgttgtgtgcctgctgaataacttctatcccagagaggccaaagtacagtggaaggtcgacaacgccctccaatcgggtaactcccaggagagtgtcacagagcaggacagcaaggacagcacctacagcctcagcagcaccctgacgctgagcaaagcagactacgagaaacacaaagtctacgcctgcgaagtcacccatcagggcctgagctcgcccgtcacaaagagcttcaacaggggagagtgttag

SEQ ID NO: 42 - protein, 213 aa, HOMO SAPIENS
EIVMTQSPATLSVSPGERATLSCRASRSIRSALAWYQHKPGQAPRLLIFGASTRATGIPARFSGSGSGTDFTLTVSSIRSEDSAVYYCQQYDFWYTFGQGTKLEIKRTVAAPSVFIFPPSDEQLKSGTASVVCLLNNFYPREAKVQWKVDNALQSGNSQESVTEQDSKDSTYSLSSTLTLSKADYEKHKVYACEVTHQGLSSPVTKSFNRGEC

SEQ ID NO: 43 - protein, 115 aa, HOMO SAPIENS
QVQLQQWGAGLLKPSETLSLTCAVYGGSFSGYYWSWIRQSPETGLEWLGEFDLGGSITHSRGTNYNPSLKSRVTISGDTSKNQFSLKLTSVTAADTAVYYCARGLAMGGTKEFDS

SEQ ID NO: 44 - protein, 96 aa, HOMO SAPIENS
DIQMTQSPDSLSASVGDRITITCRASQSINSNLAWYQQKPGKAPKLLIYKASDLESGVPSRFSGSGSGTEFTLTISSLQPDDFATYYCQQYKAFKT

SEQ ID NO: 45 - DNA, 379 bp, HOMO SAPIENS
caggtgcagctacagcagtggggcgcaggactgttgaagccttcggagaccctgtccctcacctgcgctgtctatggtgggtccttcagtggttactactggagctggatccgccagtccccagagacggggctggagtggcttggcgaattcgatcttggtggaagcatcactcatagtagaggcaccaactacaacccgtcgctcaagagtcgagtcaccatctcaggagacacgtccaagaaccagttctccctgaaactgacctctgtgaccgccgcggacacggctgtctattactgtgcgagaggtttagcaatgggtggaactaaggagtttgactcctggggccagggaaccctggtcaccgtctcctcag

SEQ ID NO: 46 - DNA, 319 bp, HOMO SAPIENS
gacatccagatgacccagtctccagactccctgtctgcatctgtaggagacagaatcaccatcacttgccgggccagtcagagtattaatagtaatttggcctggtatcagcagaaaccggggaaagcccctaagctcctgatctataaggcgtctgatttagaaagtggggtcccatcaaggttcagcggcagtggatctgggacagaattcactctcaccatcagcagcctgcagcctgatgattttgcaacttattattgccaacagtataaagcattcaagacgttcggccacgggaccaaggtggaaatcaaac

SEQ ID NO: 47 - protein, 111 aa, HOMO SAPIENS
EVQLLESGPGLVRPWGTLSLTCAVSGGSINTNNWWSWVRQSPGKGLEWIGEIHRHGDTNYNPSLKRRVSISMDESMNQFSLRLISVTAADTAVYYCCPLGYCSGDDCHRVA

SEQ ID NO: 48 - protein, 103 aa, HOMO SAPIENS
DIQMTQSPSSLSVSLGERATINCKSSQNVLDSANNRNYFGWYQQKPGQPPKLLISWASTRESGVPDRFSGSGSGTDFTLIISGLQVEDVAVYYCTQYHRLPHT

SEQ ID NO: 49 - DNA, 367 bp, HOMO SAPIENS
gaggtgcagctcttggagtcgggcccaggactggtgaggccttgggggactctgtccctcacctgcgctgtctctggtggctccatcaatactaataactggtggagttgggtccgccagtccccggggaaggggctggagtggattggagaaatccatcgtcatggggacaccaactacaacccgtcactcaagaggcgagtctccatatcgatggacgagtccatgaaccagttctccctgaggcttatctctgtgaccgccgcggacacggccgtgtattactgttgtcccctaggatattgtagtggtgatgactgtcaccgagttgcctggggccggggaatcctggtcaccgtctcttcag

SEQ ID NO: 50 - DNA, 340 bp, HOMO SAPIENS
gacatccagatgacccagtctccatcctccctgtctgtgtctctgggcgagagggccaccatcaactgcaagtccagccagaatgttttagacagcgccaacaataggaactacttcggttggtaccagcagaaaccagggcagcctcctaagctgctcatttcctgggcatctacacgggaatccggggtccctgaccgattcagtggcagcggctctgggacagacttcactctcatcatcagcggcctgcaggttgaagatgtggcagtttattactgtacacagtatcatagacttcctcacaccttcggccaagggacacgactggaaattaaac